European Patent Application EP 4 789 728 A2, published August 12, 2026. Title: PEPTIDES AND METHODS OF USING THE SAME. Applicant: SERPIN PHARMA, LLC. Application EP. The sequence listing filed with the application follows.

SEQUENCE LISTING (46 sequences)

SEQ ID NO: 1 - protein, 9 aa, Homo sapiens
FNKPFVFLM

SEQ ID NO: 2 - protein, 17 aa, Homo sapiens
VKFNKPFVFLMIEQNTK

SEQ ID NO: 3 - protein, 5 aa, Homo sapiens
FVFLM

SEQ ID NO: 4 - skipped

SEQ ID NO: 5 - protein, 9 aa, synthetic construct
  REGION 1..9: note = peptide derivative
  MOD_RES 9: note = Nle
FNKPFVFLX

SEQ ID NO: 6 - protein, 9 aa, synthetic construct
  REGION 1..9: note = peptide derivative
FNRPFLVVI

SEQ ID NO: 7 - protein, 9 aa, synthetic construct
  REGION 1..9: note = peptide derivative
  MOD_RES 9: note = Nle
FNRPFLVVX

SEQ ID NO: 8 - protein, 9 aa, synthetic construct
  REGION 1..9: note = peptide derivative
FNRPFLMII

SEQ ID NO: 9 - protein, 9 aa, synthetic construct
  REGION 1..9: note = peptide derivative
  MOD_RES 9: note = Nle
FNRPFLVIX

SEQ ID NO: 10 - protein, 5 aa, synthetic construct
  REGION 1..5: note = peptide derivative
  MOD_RES 5: note = Nle
FVFLX

SEQ ID NO: 11 - protein, 5 aa, synthetic construct
  REGION 1..5: note = peptide derivative
FLVVI

SEQ ID NO: 12 - protein, 5 aa, synthetic construct
  REGION 1..5: note = peptide derivative
  MOD_RES 5: note = Nle
FLVVX

SEQ ID NO: 13 - protein, 5 aa, synthetic construct
  REGION 1..5: note = peptide derivative
FLMII

SEQ ID NO: 14 - protein, 5 aa, synthetic construct
  REGION 1..5: note = peptide derivative
  MOD_RES 5: note = Nle
FLMIX

SEQ ID NO: 15 - skipped

SEQ ID NO: 16 - protein, 31 aa, synthetic construct
  REGION 1..31: note = peptide derivative
  SITE 1: note = MISC_FEATURE - X=any basic amino acid or absent
  SITE 2: note = MISC_FEATURE - X=any basic amino acid or absent
  SITE 3: note = MISC_FEATURE - X=any basic amino acid or absent
  SITE 4: note = MISC_FEATURE - X=any basic amino acid or absent
  SITE 5: note = MISC_FEATURE - X=any basic amino acid or absent
  SITE 6: note = MISC_FEATURE - X=any basic amino acid or absent
  SITE 7: note = MISC_FEATURE - X=any basic amino acid or absent
  SITE 8: note = MISC_FEATURE - X=any basic amino acid or absent
  SITE 9: note = MISC_FEATURE - X=any basic amino acid or absent
  SITE 10: note = MISC_FEATURE - X=any basic amino acid
  SITE 12: note = MISC_FEATURE - X=R or F
  SITE 14: note = MISC_FEATURE - X=K or R
  SITE 17: note = MISC_FEATURE - X=V or L
  SITE 18: note = MISC_FEATURE - X=F, V or M
  SITE 19: note = MISC_FEATURE - X=L, V or I
  SITE 20: note = MISC_FEATURE - X=M, I, or Nle
  SITE 22: note = MISC_FEATURE - X=any basic amino acid
  SITE 23: note = MISC_FEATURE - X=any basic amino acid or absent
  SITE 24: note = MISC_FEATURE - X=any basic amino acid or absent
  SITE 25: note = MISC_FEATURE - X=any basic amino acid or absent
  SITE 26: note = MISC_FEATURE - X=any basic amino acid or absent
  SITE 27: note = MISC_FEATURE - X=any basic amino acid or absent
  SITE 28: note = MISC_FEATURE - X=any basic amino acid or absent
  SITE 29: note = MISC_FEATURE - X=any basic amino acid or absent
  SITE 30: note = MISC_FEATURE - X=any basic amino acid or absent
  SITE 31: note = MISC_FEATURE - X=any basic amino acid or absent
XXXXXXXXXXRXNXPFXXXXRXXXXXXXXXX

SEQ ID NO: 17 - protein, 31 aa, synthetic construct
  REGION 1..31: note = peptide derivative
  SITE 1: note = MISC_FEATURE - X=any basic amino acid or absent
  SITE 2: note = MISC_FEATURE - X=any basic amino acid or absent
  SITE 3: note = MISC_FEATURE - X=any basic amino acid or absent
  SITE 4: note = MISC_FEATURE - X=any basic amino acid or absent
  SITE 5: note = MISC_FEATURE - X=any basic amino acid or absent
  SITE 6: note = MISC_FEATURE - X=any basic amino acid or absent
  SITE 7: note = MISC_FEATURE - X=any basic amino acid or absent
  SITE 8: note = MISC_FEATURE - X=any basic amino acid or absent
  SITE 9: note = MISC_FEATURE - X=any basic amino acid or absent
  SITE 10: note = MISC_FEATURE - X=any basic amino acid
  SITE 22: note = MISC_FEATURE - X=any basic amino acid
  SITE 23: note = MISC_FEATURE - X=any basic amino acid or absent
  SITE 24: note = MISC_FEATURE - X=any basic amino acid or absent
  SITE 25: note = MISC_FEATURE - X=any basic amino acid or absent
  SITE 26: note = MISC_FEATURE - X=any basic amino acid or absent
  SITE 27: note = MISC_FEATURE - X=any basic amino acid or absent
  SITE 28: note = MISC_FEATURE - X=any basic amino acid or absent
  SITE 29: note = MISC_FEATURE - X=any basic amino acid or absent
  SITE 30: note = MISC_FEATURE - X=any basic amino acid or absent
  SITE 31: note = MISC_FEATURE - X=any basic amino acid or absent
XXXXXXXXXXRFNRPFLVVIRXXXXXXXXXX

SEQ ID NO: 18 - protein, 31 aa, synthetic construct
  REGION 1..31: note = peptide derivative
  SITE 1: note = MISC_FEATURE - X=any basic amino acid or absent
  SITE 2: note = MISC_FEATURE - X=any basic amino acid or absent
  SITE 3: note = MISC_FEATURE - X=any basic amino acid or absent
  SITE 4: note = MISC_FEATURE - X=any basic amino acid or absent
  SITE 5: note = MISC_FEATURE - X=any basic amino acid or absent
  SITE 6: note = MISC_FEATURE - X=any basic amino acid or absent
  SITE 7: note = MISC_FEATURE - X=any basic amino acid or absent
  SITE 8: note = MISC_FEATURE - X=any basic amino acid or absent
  SITE 9: note = MISC_FEATURE - X=any basic amino acid or absent
  SITE 10: note = MISC_FEATURE - X=any basic amino acid
  SITE 22: note = MISC_FEATURE - X= any basic amino acid
  SITE 23: note = MISC_FEATURE - X= any basic amino acid or absent
  SITE 24: note = MISC_FEATURE - X= any basic amino acid or absent
  SITE 25: note = MISC_FEATURE - X= any basic amino acid or absent
  SITE 26: note = MISC_FEATURE - X= any basic amino acid or absent
  SITE 27: note = MISC_FEATURE - X= any basic amino acid or absent
  SITE 28: note = MISC_FEATURE - X= any basic amino acid or absent
  SITE 29: note = MISC_FEATURE - X= any basic amino acid or absent
  SITE 30: note = MISC_FEATURE - X= any basic amino acid or absent
  SITE 31: note = MISC_FEATURE - X= any basic amino acid or absent
XXXXXXXXXXRFNRPFLMIIRXXXXXXXXXX

SEQ ID NO: 19 - protein, 31 aa, synthetic construct
  REGION 1..31: note = peptide derivative
  SITE 1: note = MISC_FEATURE - X=any basic amino acid or absent
  SITE 2: note = MISC_FEATURE - X=any basic amino acid or absent
  SITE 3: note = MISC_FEATURE - X=any basic amino acid or absent
  SITE 4: note = MISC_FEATURE - X=any basic amino acid or absent
  SITE 5: note = MISC_FEATURE - X=any basic amino acid or absent
  SITE 6: note = MISC_FEATURE - X=any basic amino acid or absent
  SITE 7: note = MISC_FEATURE - X=any basic amino acid or absent
  SITE 8: note = MISC_FEATURE - X=any basic amino acid or absent
  SITE 9: note = MISC_FEATURE - X=any basic amino acid or absent
  SITE 10: note = MISC_FEATURE - X=any basic amino acid
  MOD_RES 20: note = Nle
  SITE 22: note = MISC_FEATURE - X=any basic amino acid
  SITE 23: note = MISC_FEATURE - X=any basic amino acid or absent
  SITE 24: note = MISC_FEATURE - X=any basic amino acid or absent
  SITE 25: note = MISC_FEATURE - X=any basic amino acid or absent
  SITE 26: note = MISC_FEATURE - X=any basic amino acid or absent
  SITE 27: note = MISC_FEATURE - X=any basic amino acid or absent
  SITE 28: note = MISC_FEATURE - X=any basic amino acid or absent
  SITE 29: note = MISC_FEATURE - X=any basic amino acid or absent
  SITE 30: note = MISC_FEATURE - X=any basic amino acid or absent
  SITE 31: note = MISC_FEATURE - X=any basic amino acid or absent
XXXXXXXXXXKFNKPFVFLXRXXXXXXXXXX

SEQ ID NO: 20 - protein, 16 aa, synthetic construct
  REGION 1..16: note = peptide derivative
  SITE 1: note = MISC_FEATURE - X=V or L
  SITE 2: note = MISC_FEATURE - X=any amino acid
  SITE 3: note = MISC_FEATURE - X=R or F
  SITE 4: note = MISC_FEATURE - X=any amino acid
  SITE 5: note = MISC_FEATURE - X=R or K
  SITE 6: note = MISC_FEATURE - X=any amino acid
  SITE 11: note = MISC_FEATURE - X=M, Nle, or I
  SITE 12: note = MISC_FEATURE - X=any amino acid
  SITE 13: note = MISC_FEATURE - X=any amino acid
  SITE 14: note = MISC_FEATURE - X=any amino acid
  SITE 15: note = MISC_FEATURE - X=any amino acid
  SITE 16: note = MISC_FEATURE - X=any amino acid
XXXXXXFVFLXXXXXX

SEQ ID NO: 21 - skipped

SEQ ID NO: 22 - protein, 21 aa, synthetic construct
  REGION 1..21: note = peptide derivative
FPKMVPQFNTELKIFPEVNIK

SEQ ID NO: 23 - protein, 33 aa, Homo sapiens
SIPPEVKFNKPFVFLMIEQNTKSPLFMGKVVNP

SEQ ID NO: 24 - protein, 17 aa, Homo sapiens
VKFNKPFVFLMIEQNTK

SEQ ID NO: 25 - protein, 11 aa, Homo sapiens
VKFNKPFVFLM

SEQ ID NO: 26 - protein, 23 aa, synthetic construct
  REGION 1..23: note = peptide derivative
RRRVKFNKPFVFLMIEQNTKRRR

SEQ ID NO: 27 - protein, 17 aa, synthetic construct
  REGION 1..17: note = peptide derivative
RRRVKFNKPFVFLMRRR

SEQ ID NO: 28 - protein, 17 aa, synthetic construct
  REGION 1..17: note = peptide derivative
LRFNRPFLVVIFSTSTQ

SEQ ID NO: 29 - protein, 11 aa, synthetic construct
  REGION 1..11: note = peptide derivative
LRFNRPFLVVI

SEQ ID NO: 30 - protein, 17 aa, synthetic construct
  REGION 1..17: note = peptide derivative
RRRLRFNRPFLVVIRRR

SEQ ID NO: 31 - protein, 11 aa, synthetic construct
  REGION 1..11: note = peptide derivative
VRFNRPFLMII

SEQ ID NO: 32 - protein, 17 aa, synthetic construct
  REGION 1..17: note = peptide derivative
RRRVRFNRPFLMIIRRR

SEQ ID NO: 33 - protein, 8 aa, synthetic construct
  REGION 1..8: note = peptide derivative
VRFNRPFL

SEQ ID NO: 34 - protein, 14 aa, synthetic construct
  REGION 1..14: note = peptide derivative
RRRVRFNRPFLRRR

SEQ ID NO: 35 - protein, 17 aa, synthetic construct
  REGION 1..17: note = peptide derivative
  MOD_RES 11: note = Nle
VKFNKPFVFLXIEQNTK

SEQ ID NO: 36 - protein, 17 aa, synthetic construct
  REGION 1..17: note = peptide derivative
VKFNKAAAAAAIEQNTK

SEQ ID NO: 37 - protein, 31 aa, synthetic construct
  REGION 1..31: note = peptide derivative
  SITE 1: note = MISC_FEATURE - X=any amino acid or absent
  SITE 2: note = MISC_FEATURE - X=any amino acid or absent
  SITE 3: note = MISC_FEATURE - X=any amino acid or absent
  SITE 4: note = MISC_FEATURE - X=any amino acid or absent
  SITE 5: note = MISC_FEATURE - X=any amino acid or absent
  SITE 6: note = MISC_FEATURE - X=any amino acid or absent
  SITE 7: note = MISC_FEATURE - X=any amino acid or absent
  SITE 8: note = MISC_FEATURE - X=any amino acid or absent
  SITE 9: note = MISC_FEATURE - X=any amino acid or absent
  SITE 10: note = MISC_FEATURE - X=any amino acid
  MOD_RES 20: note = Nle
  SITE 22: note = MISC_FEATURE - X=any amino acid or absent
  SITE 23: note = MISC_FEATURE - X=any amino acid or absent
  SITE 24: note = MISC_FEATURE - X=any amino acid or absent
  SITE 25: note = MISC_FEATURE - X=any amino acid or absent
  SITE 26: note = MISC_FEATURE - X=any amino acid or absent
  SITE 27: note = MISC_FEATURE - X=any amino acid or absent
  SITE 28: note = MISC_FEATURE - X=any amino acid or absent
  SITE 29: note = MISC_FEATURE - X=any amino acid or absent
  SITE 30: note = MISC_FEATURE - X=any amino acid or absent
  SITE 31: note = MISC_FEATURE - X=any amino acid or absent
XXXXXXXXXXRFNKPFVFLXRXXXXXXXXXX

SEQ ID NO: 38 - protein, 11 aa, synthetic construct
  REGION 1..11: note = peptide derivative
VKFNKPFVFLM

SEQ ID NO: 39 - protein, 11 aa, synthetic construct
  REGION 1..11: note = peptide derivative
LRFNRPFLVVI

SEQ ID NO: 40 - protein, 11 aa, synthetic construct
  REGION 1..11: note = peptide derivative
  MOD_RES 11: note = Nle
VKFNKPFVFLX

SEQ ID NO: 41 - protein, 11 aa, synthetic construct
  REGION 1..11: note = peptide derivative
RFNRPFLVVIR

SEQ ID NO: 42 - protein, 11 aa, synthetic construct
  REGION 1..11: note = peptide derivative
RFNRPFLMIIR

SEQ ID NO: 43 - protein, 11 aa, synthetic construct
  REGION 1..11: note = peptide derivative
  MOD_RES 10: note = Nle
RFNKPFVFLXR

SEQ ID NO: 44 - protein, 11 aa, synthetic construct
  REGION 1..11: note = peptide derivative
RRRFLVVIRRR

SEQ ID NO: 45 - protein, 11 aa, synthetic construct
  REGION 1..11: note = peptide derivative
RRRFLMIIRRR

SEQ ID NO: 46 - protein, 11 aa, synthetic construct
  REGION 1..11: note = peptide derivative
  MOD_RES 8: note = Nle
RRRFVFLXRRR